European Patent Specification EP 3 555 135 B1, published April 10, 2024. Title: IL-11Ralpha Antibodies. Applicant: Singapore Health Services Pte. Ltd National University of Singapore Clegg, Richard I. The sequence listing filed with the application follows.

SEQUENCE LISTING (99 sequences)

SEQ ID NO: 1 - protein, 112 aa, Artificial Sequence
  BSO-1E3_1
DVVMTQIPLSLSVSMKFQASISCRSSQSLVHSNGNTYLHWYLQKPGQSPKLLIYKVSNRFSGVPDRFSGSGSGTDFTLKISRVEAEDLGVYFCSQSTHVPLTFGAGTKLELK

SEQ ID NO: 2 - protein, 107 aa, Artificial Sequence
  BSO-1E3_2
NIVMTQSPKSMSMSVGERVTLSCKASENVGTYVSWYQQKPEQSPKLLIYGASNRYTGVPDRFTGSGSATDFTLTISSVQAEDLADYHCGQGYSYPYTFGGGTKLEIK

SEQ ID NO: 3 - protein, 107 aa, Artificial Sequence
  BSO-2E5
DIQMTQSPSSLSASLGERVSLTCRASQDIGSSLNWLQQEPDGTIKRLIYATASLESGVPKRFSGSRSGSDYSLTISRLESEDFVDYYCQQYASSPPTFGAGTKLELK

SEQ ID NO: 4 - protein, 111 aa, Artificial Sequence
  BSO-4G3
DIVLTQSPASLAVSLGQSVTISCRASESVEYSGTTLMQWYQQKPGQPPKLLIYGASNVESGVPARFSGSGSGTDFSLNIHPVEEDDIAMYFCQQSRKVPYTFGSGTKLEIK

SEQ ID NO: 5 - protein, 113 aa, Artificial Sequence
  BSO-5E5
DIVMSQSPSSLPVSVGENVTMSCKSSQSLLYGSNQKNYLAWYQQKPGQSPKLLIYWASTRESGVPDRFTGSGSGTDFTLTISSVKAEDLAVYFCQQYYSYPRTFGGGTKLEIK

SEQ ID NO: 6 - protein, 112 aa, Artificial Sequence
  BSO-7G9
DVVMTQTPLSLPVSLGDQASISCRSSQSLVHSNGNTYLHWYLQKPGQSPKLLIYKVSNRFSGVPDRFSGSGSGTDFTLKISRVEAEDLGVYFCSQSTHVPLTFGAGTKLELK

SEQ ID NO: 7 - protein, 107 aa, Artificial Sequence
  BSO-9A7
DIVLTQSPATLSMTPGDSVSLSCRASQSISNNLHWYQQKSHESPRLLIKYASQSISGIPSRFSGSGSGTDFTLSFNSVETEDFGVYFCQQRYSWPLTFGAGTKLEMK

SEQ ID NO: 8 - protein, 107 aa, Artificial Sequence
  BSO-10D11
DIQMTQSPSSLSASLGERVSLTCRASQEISAYLSWLQQKPDGTIKRLIYSTSTLDSGVPKRFSGSRSGSDYSLTISSLESEDFADYFCLQYASSPLTFGAGTKLELK

SEQ ID NO: 9 - protein, 107 aa, Artificial Sequence
  BSO-13B10
DIVMTQSQKFMSTSVGDRVSVTCKASQNVGSNVAWYQQKAGQSPKALIYSASYRYSGVPDRFTGSGSGTDFTLTISNVQSEDLAEYFCQQYNSYPLTFGAGTKLELK

SEQ ID NO: 10 - protein, 119 aa, Artificial Sequence
  BSO-1E3_1
QVQLQQPGAELVTPGASVKLSCKASGFTFTNNWMHWVKQRPGQGLEWIGMIHPNSGITNINEKFKNKATVTVDKSSSTVYIQLSSLTSEDSAVYYCRSDGTYEGYFDYWGQGTPLTVSS

SEQ ID NO: 11 - protein, 117 aa, Artificial Sequence
  BSO-1E3_2
QVQLQQSGPELVKPGASVKISCKASGYNFNDYYINWVNQRPGQGLEWIGWIFPGRIITYYNEKFKGKATLTVDTSSNTAYMLLSSLTSEDSAVYFCARGVGEGFDYWGQGTTLTVSS

SEQ ID NO: 12 - protein, 113 aa, Artificial Sequence
  BSO-2E5
QGQVQQSGAELVKPGASVKLSCKTSGFTFSTSYISWLKQKPRQSLEWIAWIYAGTGSTSYNQKFTGKAQLTVDTSSSTAYMQLSSLTSEDSAIYYCARHWAYWGQGTLVTVSA

SEQ ID NO: 13 - protein, 115 aa, Artificial Sequence
  BSO-4G3
EVQLVESGGGLVKPGGSLKLSCAASGFTFSTYAMSWVRQTPEKRLEWVAAIKSNGGSTYYPDTVKDRFTISRDNAKNTLYLQMSSLRPEDTALYYCAHGLLFAHWGQGTLVTVSA

SEQ ID NO: 14 - protein, 122 aa, Artificial Sequence
  BSO-5E5
DVQLQESGPGLVKPSQSLSLTCSVTGYSITSDYYWNWIRQFPGNKLEWMGYISYDSSNNYNPSLKNRISITRDTSKNQFFLKLNSVTTEDTATYYCASVGYYYVSDWYFDVWGTGTTVTVSS

SEQ ID NO: 15 - protein, 122 aa, Artificial Sequence
  BSO-7G9
QVQLQQPGAELVKPGASVRLSCKASGYTFTSYWMHWVKQRPGQGLEWIGMIHPNSGYTNYNEKFKIKATLTVDKSSSTAHMQLSSLTSEDSAVYHCARGGYDGSYGPWFAYWGQGTLVTVSA

SEQ ID NO: 16 - protein, 117 aa, Artificial Sequence
  BSO-9A7
QVQLQQPGAELVRPGSSVKLSCKASGYTFTNYWMHWLKQRPVQGLEWIGNIGPSDSKTHYNQKFKDKATLTVDKSSSTAYMQLNSLTSEDSAVYYCARGDYVLFTYWGQGTLVTVSA

SEQ ID NO: 17 - protein, 121 aa, Artificial Sequence
  BSO-10D11
QVQLQQSGTELVRPGTSVKMSCKAAGYTFTDYWIGWIKQRPGHGLEWIGDIFPGGDYTKCSERFKGKAKLTADTSSSTAYMQLSRLTSEDSAIYYCARRSTTIRFGAMDNWGQGTSVTVSS

SEQ ID NO: 18 - protein, 118 aa, Artificial Sequence
  BSO-13B10
QVQLKESGPGLVAPSQSLSITCTVSGFSLTSFSISWVRQPPGKGLEWLGGIWTGGGTNYNSALKPRLSISKDNSKSQVFLKMNSLQTDDTARYYCARNSNYPSGFAYWGQGTLVTVSA

SEQ ID NO: 19 - protein, 11 aa, Artificial Sequence
  BSO-1E3_1 CDR1 Light Chain
QSLVHSNGNTY

SEQ ID NO: 20 - protein, 3 aa, Artificial Sequence
  BSO-1E3_1 CDR2 Light Chain
KVS

SEQ ID NO: 21 - protein, 9 aa, Artificial Sequence
  BSO-1E3_1 CDR3 Light Chain
SQSTHVPLT

SEQ ID NO: 22 - protein, 6 aa, Artificial Sequence
  BSO-1E3_2 CDR1 Light Chain
ENVGTY

SEQ ID NO: 23 - protein, 3 aa, Artificial Sequence
  BSO-1E3_2 CDR2 Light Chain
GAS

SEQ ID NO: 24 - protein, 9 aa, Artificial Sequence
  BSO-1E3_2 CDR3 Light Chain
GQGYSYPYT

SEQ ID NO: 25 - protein, 6 aa, Artificial Sequence
  BSO-2E5 CDR1 Light Chain
QDIGSS

SEQ ID NO: 26 - protein, 3 aa, Artificial Sequence
  BSO-2E5 CDR2 Light Chain
ATA

SEQ ID NO: 27 - protein, 9 aa, Artificial Sequence
  BSO-2E5 CDR3 Light Chain
QQYASSPPT

SEQ ID NO: 28 - protein, 10 aa, Artificial Sequence
  BSO-4G3 CDR1 Light Chain
ESVEYSGTTL

SEQ ID NO: 29 - protein, 9 aa, Artificial Sequence
  BSO-4G3 CDR3 Light Chain
QQSRKVPYT

SEQ ID NO: 30 - protein, 12 aa, Artificial Sequence
  BSO-5E5 CDR1 Light Chain
QSLLYGSNQKNY

SEQ ID NO: 31 - protein, 3 aa, Artificial Sequence
  BSO-5E5 CDR2 Light Chain
WAS

SEQ ID NO: 32 - protein, 9 aa, Artificial Sequence
  BSO-5E5 CDR3 Light Chain
QQYYSYPRT

SEQ ID NO: 33 - protein, 6 aa, Artificial Sequence
  BSO-9A7 CDR1 Light Chain
QSISNN

SEQ ID NO: 34 - protein, 3 aa, Artificial Sequence
  BSO-9A7 CDR2 Light Chain
YAS

SEQ ID NO: 35 - protein, 9 aa, Artificial Sequence
  BSO-9A7 CDR3 Light Chain
QQRYSWPLT

SEQ ID NO: 36 - protein, 6 aa, Artificial Sequence
  BSO-10D11 CDR1 Light Chain
QEISAY

SEQ ID NO: 37 - protein, 3 aa, Artificial Sequence
  BSO-10D11 CDR2 Light Chain
STS

SEQ ID NO: 38 - protein, 9 aa, Artificial Sequence
  BSO-10D11 CDR3 Light Chain
LQYASSPLT

SEQ ID NO: 39 - protein, 6 aa, Artificial Sequence
  BSO-13B10 CDR1 Light Chain
QNVGSN

SEQ ID NO: 40 - protein, 3 aa, Artificial Sequence
  BSO-13B10 CDR2 Light Chain
SAS

SEQ ID NO: 41 - protein, 9 aa, Artificial Sequence
  BSO-13B10 CDR3 Light Chain
QQYNSYPLT

SEQ ID NO: 42 - protein, 8 aa, Artificial Sequence
  BSO-1E3_1 CDR1 Heavy Chain
GFTFTNNW

SEQ ID NO: 43 - protein, 8 aa, Artificial Sequence
  BSO-1E3_1 CDR2 Heavy Chain
IHPNSGIT

SEQ ID NO: 44 - protein, 12 aa, Artificial Sequence
  BSO-1E3_1 CDR3 Heavy Chain
RSDGTYEGYFDY

SEQ ID NO: 45 - protein, 8 aa, Artificial Sequence
  BSO-1E3_2 CDR1 Heavy Chain
GYNFNDYY

SEQ ID NO: 46 - protein, 8 aa, Artificial Sequence
  BSO-1E3_2 CDR2 Heavy Chain
IFPGRIIT

SEQ ID NO: 47 - protein, 10 aa, Artificial Sequence
  BSO-1E3_1 CDR3 Heavy Chain
ARGVGEGFDY

SEQ ID NO: 48 - protein, 8 aa, Artificial Sequence
  BSO 2E5 CDR1 Heavy Chain
GFTFSTSY

SEQ ID NO: 49 - protein, 8 aa, Artificial Sequence
  BSO-2E5 CDR2 Heavy Chain
IYAGTGST

SEQ ID NO: 50 - protein, 6 aa, Artificial Sequence
  BSO-2E5 CDR3 Heavy Chain
ARHWAY

SEQ ID NO: 51 - protein, 8 aa, Artificial Sequence
  BSO-4G3 CDR1 Heavy Chain
GFTFSTYA

SEQ ID NO: 52 - protein, 8 aa, Artificial Sequence
  BSO-4G3 CDR2 Heavy Chain
IKSNGGST

SEQ ID NO: 53 - protein, 8 aa, Artificial Sequence
  BSO-4G3 CDR3 Heavy Chain
AHGLLFAH

SEQ ID NO: 54 - protein, 9 aa, Artificial Sequence
  BSO-5E5 CDR1 Heavy Chain
GYSITSDYY

SEQ ID NO: 55 - protein, 7 aa, Artificial Sequence
  BSO-5E5 CDR2 Heavy Chain
ISYDSSN

SEQ ID NO: 56 - protein, 15 aa, Artificial Sequence
  BSO-5E5 CDR3 Heavy Chain
ASVGYYYVSDWYFDV

SEQ ID NO: 57 - protein, 8 aa, Artificial Sequence
  BSO-7G9 CDR1 Heavy Chain
GYTFTSYW

SEQ ID NO: 58 - protein, 8 aa, Artificial Sequence
  BSO-7G9 CDR2 Heavy Chain
IHPNSGYT

SEQ ID NO: 59 - protein, 15 aa, Artificial Sequence
  BSO-7G9 CDR3 Heavy Chain
ARGGYDGSYGPWFAY

SEQ ID NO: 60 - protein, 8 aa, Artificial Sequence
  BSO-9A7 CDR1 Heavy Chain
GYTFTNYW

SEQ ID NO: 61 - protein, 8 aa, Artificial Sequence
  BSO-9A7 CDR2 Heavy Chain
IGPSDSKT

SEQ ID NO: 62 - protein, 10 aa, Artificial Sequence
  BSO-9A7 CDR3 Heavy Chain
ARGDYVLFTY

SEQ ID NO: 63 - protein, 8 aa, Artificial Sequence
  BSO-10D11 CDR1 Heavy Chain
GYTFTDYW

SEQ ID NO: 64 - protein, 8 aa, Artificial Sequence
  BSO-10D11 CDR2 Heavy Chain
IFPGGDYT

SEQ ID NO: 65 - protein, 14 aa, Artificial Sequence
  BSO-10D11 CDR3 Heavy Chain
ARRSTTIRFGAMDN

SEQ ID NO: 66 - protein, 8 aa, Artificial Sequence
  BSO-13B10 CDR1 Heavy Chain
GFSLTSFS

SEQ ID NO: 67 - protein, 7 aa, Artificial Sequence
  BSO-13B10 CDR2 Heavy Chain
IWTGGGT

SEQ ID NO: 68 - protein, 12 aa, Artificial Sequence
  BSO-13B10 CDR3 Heavy Chain
ARNSNYPSGFAY

SEQ ID NO: 69 - protein, 6 aa, Artificial Sequence
  BSO-9A7, BSO-10D11, BSO-13B10, BSO-2E5 LC-CDR1-1 Family consensus
  MISC_FEATURE (2)..(2): X = N, S, E or D
  MISC_FEATURE (3)..(3): X = I or V
  MISC_FEATURE (4)..(4): X = G or S
  MISC_FEATURE (5)..(5): X = S, N or A
  MISC_FEATURE (6)..(6): X = N, Y or S
QXXXXX

SEQ ID NO: 70 - protein, 12 aa, Artificial Sequence
  BSO-5E5, BSO-1E3_1, BSO-7G9 LC-CDR1-2 Family Consensus
  MISC_FEATURE (4)..(4): X = Absent or L
  MISC_FEATURE (5)..(5): X = V or Y
  MISC_FEATURE (6)..(6): X = H or G
  MISC_FEATURE (9)..(9): X = G or Q
  MISC_FEATURE (10)..(10): X = N or K
  MISC_FEATURE (11)..(11): X = T or N
QSLXXXSNXXXY

SEQ ID NO: 71 - protein, 3 aa, Artificial Sequence
  BSO-4G3, BSO-1E3_2, BSO-5E5, BSO-9A7, BSO-13B10 LC-CDR2-1 Family Consensus
  MISC_FEATURE (1)..(1): X = G, W, Y or S
XAS

SEQ ID NO: 72 - protein, 3 aa, Artificial Sequence
  BSO-10D11, BSO-1E3_1, BSO-7G9 LC-CDR2-2 Family Consensus
  MISC_FEATURE (1)..(1): X = S or K
  MISC_FEATURE (2)..(2): X = T or V
XXS

SEQ ID NO: 73 - protein, 9 aa, Artificial Sequence
  BSO-1E3_1, BSO-7G9, BSO-1E3_2, BSO-2E5, BSO-4G3, BSO-5E5, BSO-9A7, BSO-10D11, BSo-13B10 LC-CDR3-1 Family Consensus
  MISC_FEATURE (1)..(1): X = Q, S, G or L
  MISC_FEATURE (3)..(3): X = Y, S, G or R
  MISC_FEATURE (4)..(4): X = Y, A, T, N or R
  MISC_FEATURE (5)..(5): X = S, H or K
  MISC_FEATURE (6)..(6): X = V, Y, S or W
  MISC_FEATURE (8)..(8): X = L, Y, R or P
XQXXXXPXT

SEQ ID NO: 74 - protein, 8 aa, Artificial Sequence
  BSO-7G9, BSO-9A7, BSO-10D11 HC-CDR1-1 Family Consensus
  MISC_FEATURE (6)..(6): X = S, N or D
GYTFTXYW

SEQ ID NO: 75 - protein, 8 aa, Artificial Sequence
  BSO-2E5, BSO-4G3, BSO-1E3_1 HC-CDR1-2 Family Consensus
  MISC_FEATURE (5)..(5): X = S or T
  MISC_FEATURE (6)..(6): X = T or N
  MISC_FEATURE (7)..(7): X = S, Y or N
  MISC_FEATURE (8)..(8): X = Y, A or W
GFTFXXXX

SEQ ID NO: 76 - protein, 9 aa, Artificial Sequence
  BSO-5E5, BSO-1E3_2 HC-CDR1-3 Family Consensus
  MISC_FEATURE (3)..(3): X = S or N
  MISC_FEATURE (4)..(4): X = I or F
  MISC_FEATURE (5)..(5): X = T or N
  MISC_FEATURE (6)..(6): X = Absent or S
GYXXXXDYY

SEQ ID NO: 77 - protein, 8 aa, Artificial Sequence
  BSO-1E3_1, BSO-4G3, BSO-2E5, BSO-7G9 HC-CDR2-1 Family Consensus
  MISC_FEATURE (2)..(2): X = H, K or Y
  MISC_FEATURE (3)..(3): X = P, S or A
  MISC_FEATURE (4)..(4): X = N or G
  MISC_FEATURE (5)..(5): X = S, G or T
  MISC_FEATURE (7)..(7): X = S, I or Y
IXXXXGXT

SEQ ID NO: 78 - protein, 8 aa, Artificial Sequence
  BSO-1E3_2, BSO-10D11 HC-CDR2-2 Family Consensus
  MISC_FEATURE (5)..(5): X = R or G
  MISC_FEATURE (6)..(6): X = I or D
  MISC_FEATURE (7)..(7): X = I or Y
IFPGXXXT

SEQ ID NO: 79 - protein, 15 aa, Artificial Sequence
  BSO-7G9, BSO-1E3_2, BSO-9A7 HC-CDR3-1 Family Consensus
  MISC_FEATURE (4)..(4): X = Absent, D or G
  MISC_FEATURE (5)..(5): X = Absent or Y
  MISC_FEATURE (6)..(6): X = V or D
  MISC_FEATURE (7)..(7): X = G or L
  MISC_FEATURE (8)..(8): X = Absent, E or S
  MISC_FEATURE (9)..(9): X = Absent or Y
  MISC_FEATURE (10)..(10): X = Absent or G
  MISC_FEATURE (11)..(11): X = Absent or P
  MISC_FEATURE (12)..(12): X = Absent or W
  MISC_FEATURE (14)..(14): X = D, T or A
ARGXXXXXXXXXFXY

SEQ ID NO: 80 - DNA, 336 bp, Artificial Sequence
  BSO-1E3_1
gatgttgtgatgacccaaattccactctccctgtctgtcagtatgaagttccaagcctccatctcttgcagatctagtcagagccttgtacacagtaatggaaacacctatttacattggtacctgcagaagccaggccagtctccaaagctcctgatctacaaagtttccaaccgattttctggggtcccagacaggttcagtggcagtggatcagggacagatttcacactcaagatcagcagagtggaggctgaggatctgggagtttatttctgctctcaaagtacacatgttccgctcacgttcggtgctgggaccaagctggagctgaaa

SEQ ID NO: 81 - DNA, 321 bp, Artificial Sequence
  BSO-1ES_2
aacattgtaatgacccaatctcccaaatccatgtccatgtcagtaggagagagggtcaccttgagctgcaaggccagtgagaatgtgggtacttatgtatcctggtatcaacagaaaccagagcagtctcctaaactgctgatatacggggcatccaaccggtacactggggtccccgatcgcttcacaggcagtggatctgcaacagatttcactctgaccatcagcagtgtgcaggctgaagaccttgcagattatcactgtggacagggttacagctatccgtacacgttcggaggggggaccaagctggaaataaaa

SEQ ID NO: 82 - DNA, 321 bp, Artificial Sequence
  BSO-2E5
gacatccagatgacccagtctccatcctccttatctgcctctctgggagaaagagtcagtctcacttgtcgggcaagtcaggacattggtagtagcttaaactggcttcagcaggaaccagatggaactattaaacgcctgatctacgccacagccagtttagaatctggtgtccccaaaaggttcagtggcagtaggtctgggtcagactattctctcaccatcagcagacttgagtctgaagattttgtagactattactgtcaacaatatgctagctctcctcccacgttcggtgctgggaccaagctggagctgaaa

SEQ ID NO: 83 - DNA, 333 bp, Artificial Sequence
  BSO-4G3
gacattgtgctcacccaatctccagcttctttggctgtgtctctagggcagagtgtcaccatctcctgcagagccagtgaaagtgttgaatattctggcactactttaatgcagtggtaccaacagaaaccaggacagccacccaaactcctcatctatggtgcatccaacgtagaatctggggtccctgccaggtttagtggcagtgggtctgggacagacttcagcctcaacatccatcctgtggaggaggatgatattgcaatgtatttctgtcagcaaagtaggaaggttccgtatacgttcggatcggggaccaagctggaaataaaa

SEQ ID NO: 84 - DNA, 339 bp, Artificial Sequence
  BSO-5E5
gacattgtgatgtcacagtctccatcctccctacctgtgtcagttggagagaatgttactatgagctgcaagtccagtcagagccttttatatggtagcaatcaaaagaactacttggcctggtaccagcagaaaccagggcagtctcctaaactgctgatttactgggcatccactagggaatctggggtccctgatcgcttcacaggcagtggatctgggacagatttcactctcaccatcagcagtgtgaaggctgaagacctggcagtttatttctgtcagcaatattatagctatcctcggacgttcggtggaggcaccaagctggaaatcaaa

SEQ ID NO: 85 - DNA, 336 bp, Artificial Sequence
  BSO-7G9
gatgttgtgatgacccaaactccactctccctgcctgtcagtcttggagatcaagcctccatctcttgcagatctagtcagagccttgtacacagtaatggaaacacctatttacattggtacctgcagaagccaggccagtctccaaagctcctgatctacaaagtttccaaccgattttctggggtcccagacaggttcagtggcagtggatcagggacagatttcacactcaagatcagcagagtggaggctgaggatctgggagtttatttctgctctcaaagtacacatgttccgctcacgttcggtgctgggaccaagctggagctgaaa

SEQ ID NO: 86 - DNA, 321 bp, Artificial Sequence
  BSO-9A7
gatattgtgctaactcagtctccagccaccctgtctatgactccaggagatagcgtcagtctttcctgcagggccagccaaagtattagcaacaacctacactggtatcaacaaaaatcacatgagtctccaaggcttctcatcaagtatgcttcccagtccatctctgggatcccctccaggttcagtggcagtggatcggggacagatttcactctcagtttcaacagtgtggagactgaagattttggagtgtatttctgtcaacagagatacagctggcctctcacgttcggtgctgggaccaagctggaaatgaaa

SEQ ID NO: 87 - DNA, 321 bp, Artificial Sequence
  BSO-10D11
gacatccagatgacccagtctccatcctccttatctgcctctctgggagaaagagtcagtctcacttgtcgggcaagtcaggaaattagtgcttacttaagctggcttcagcagaaaccagatggaactattaaacgcctgatctacagcacatccactttagattctggtgtcccaaaaaggttcagtggcagtaggtctgggtcagattattctctcaccatcagcagccttgagtctgaagattttgcagactatttctgtctccaatatgctagttctccgctcacgttcggtgctgggaccaagctggagctgaaa

SEQ ID NO: 88 - DNA, 321 bp, Artificial Sequence
  BSO-13B10
gacattgtgatgacccagtctcaaaaattcatgtccacatcagtaggagacagggtcagcgtcacctgcaaggccagtcagaatgtgggtagtaatgtagcctggtatcaacagaaagcagggcaatctcctaaagcactgatttactcggcatcctaccggtacagtggagtccctgatcgcttcacaggcagtggatctgggacagatttcactctcaccatcagcaatgtgcagtctgaagacttggcagagtatttctgtcagcaatataacagctatccgctcacgttcggtgctgggaccaagctggagctgaaa

SEQ ID NO: 89 - DNA, 357 bp, Artificial Sequence
  BSO-1E3_1
caggtccaactgcagcagcctggggctgaactggtcacgcctggggcttcagtgaagttgtcctgcaaggcttctggcttcactttcaccaacaactggatgcactgggtgaagcagagacctggacaaggccttgagtggattggaatgattcatcctaatagtgggattactaacatcaatgagaagttcaagaacaaggccacagtgactgtagacaaatcctccagcacagtctacatacaactcagcagcctgacatctgaggactctgcggtctattactgtcgctccgatggtacctacgagggctactttgactactggggccaaggcacccctctcacagtctcctca

SEQ ID NO: 90 - DNA, 351 bp, Artificial Sequence
  BSO-1E3_2
caggtccaactacagcagtctggacctgaactggtgaagcctggggcttcagtgaagatatcctgcaaggcttctggctacaatttcaatgactactatataaactgggtgaaccagaggcctggacagggacttgagtggattggatggatttttcctggaagaattattacttactacaatgagaaattcaagggcaaggccacacttactgtagacacatcctccaacacagcctacatgttgctcagcagcctgacctctgaggactctgcggtctatttctgtgcaagaggggtaggagagggctttgactactggggccaaggcaccactctcacagtctcctca

SEQ ID NO: 91 - DNA, 339 bp, Artificial Sequence
  BSO-2E5
cagggtcaggtgcagcagtctggagctgagctggtgaagcctggggcttcagtgaagctgtcctgcaagacttctggcttcaccttcagtactagttatataagttggttgaagcagaagcctcgacagagtcttgagtggattgcatggatttatgctggaactggtagtactagctataatcagaaattcacaggcaaggcccaactgactgtagacacatcctccagcacagcctacatgcaactcagcagcctgacatctgaggactctgccatctattactgtgcaagacactgggcttactggggccaagggactctggtcactgtctctgca

SEQ ID NO: 92 - DNA, 345 bp, Artificial Sequence
  BSO-4G3
gaggtgcagctggtggagtctgggggaggcttagtgaagcctggcgggtccctgaaactctcctgtgcagcctctggattcactttcagtacctatgccatgtcttgggttcgccagactccagagaagaggctggagtgggtcgcagccattaaaagtaatggtggtagcacctactatccagacactgtgaaggaccgattcaccatttccagagacaatgccaagaacaccctgtacctgcaaatgagcagtctgaggcctgaggacacagccttgtattactgtgcacatggtctcctgtttgctcactggggccaagggactctggtcactgtctctgca

SEQ ID NO: 93 - DNA, 366 bp, Artificial Sequence
  BSO-5E5
  misc_feature (352)..(352): n is a, c, g, or t
gatgtacagcttcaggagtcaggacctggcctcgtgaaaccttctcagtctctgtctctcacctgctctgtcactggctactccatcaccagtgattattactggaactggatccggcagtttccaggaaacaaactggaatggatgggctacataagctacgatagtagcaataactacaacccatctctcaaaaatcgaatctccatcactcgtgacacatctaagaaccagtttttcctgaagttgaattctgtgactactgaggacacagccacatattactgtgcttcagtgggttattactacgttagtgactggtacttcgatgtctggggcacagggaccacgntcaccgtctcctca

SEQ ID NO: 94 - DNA, 366 bp, Artificial Sequence
  BSO-7G9
caggtccaactgcagcagcctggggctgagctggtaaagcctggggcttcagtgaggttgtcctgcaaggcttctggctacactttcaccagctactggatgcactgggtgaagcagaggcctggacaaggccttgagtggattggaatgattcatcctaatagtggttatactaattacaatgagaagttcaagatcaaggccacactgactgtagacaaatcctccagcacagcccacatgcaactcagcagcctgacatctgaggattctgcggtctatcactgtgcaagaggggggtatgatggttcctacgggccctggtttgcttactggggccaagggactctggtcactgtctctgca

SEQ ID NO: 95 - DNA, 351 bp, Artificial Sequence
  BSO-9A7
caggtccaactgcagcagcctggggctgagctggtgaggcctgggtcttcagtgaagctgtcctgcaaggcttctggctacaccttcaccaactactggatgcattggttgaagcagaggcctgtacaaggccttgagtggattggtaacattggcccttctgatagtaaaactcactacaatcaaaaattcaaggacaaggccacattgactgtagacaaatcctccagcacagcctacatgcaactcaacagcctgacatctgaggactctgcggtctattactgtgcaaggggtgattacgtcctgtttacttactggggccaagggactctggtcactgtctctgca

SEQ ID NO: 96 - DNA, 363 bp, Artificial Sequence
  BSO-10D11
caggtccagctgcagcagtctggaactgagctggtaaggcctgggacttcagtgaagatgtcctgcaaggctgctggatacaccttcactgactactggataggttggataaagcagaggcctggacatggccttgagtggattggagatattttccctggaggtgattatactaagtgcagtgagaggttcaagggcaaggccaaactgactgcagacacatcctccagcactgcctacatgcagctcagcagactgacatctgaggactctgccatctattactgtgcaagaaggagtactacgatacgcttcggggctatggacaactggggtcaaggaacctcagtcaccgtctcctca

SEQ ID NO: 97 - DNA, 354 bp, Artificial Sequence
  BSO-13B10
caggtgcagctgaaggagtcaggacctggcctggtggcgccctcacagagcctgtccatcacatgcactgtctctgggttctcattaaccagcttttctataagctgggttcgccagccaccaggaaagggtctggagtggcttggaggaatatggactggtggaggcacaaattataattcagctctcaaacccagactgagcatcagcaaagacaactccaagagtcaagttttcttaaaaatgaacagtctgcaaactgatgacacagccaggtactactgtgccagaaatagtaactacccttccgggtttgcttactggggccaagggactctggtcactgtctctgca

SEQ ID NO: 98 - DNA, 1575 bp, Artificial Sequence
  IL-11:IL-11Ralpha fusion protein
gaattcccgccgccaccatgggctggtcctgcatcatcctgtttctggtggccacagccaccggcgtgcactctccacaggcttggggacctccaggcgtgcagtatggccagcctggcagatccgtgaagctgtgctgtcctggcgtgacagctggcgaccctgtgtcctggttcagagatggcgagcccaagctgctgcagggcccagattctggactgggccacgaactggtgctggcccaggccgattctaccgacgagggcacctacatctgccagaccctggatggcgccctgggcggaacagtgacactgcagctgggctaccctcccgccagacctgtggtgtcttgtcaggccgccgactacgagaacttcagctgcacatggtcccccagccagatcagcggcctgcccaccagatacctgaccagctaccggaagaaaaccgtgctgggcgccgacagccagagaagaagcccttctacaggcccctggccctgccctcaggatcctctgggagctgccagatgtgtggtgcacggcgccgagttctggtcccagtaccggatcaacgtgaccgaagtgaaccccctgggcgcctccacaagactgctggatgtgtccctgcagagcatcctgcggcccgatcctccacagggcctgagagtggaaagcgtgcccggctaccccagaaggctgagagccagctggacataccccgcctcttggccttgccagccccacttcctgctgaagtttcggctgcagtaccggccagcccagcaccctgcttggagcacagtggaacctgccggcctggaagaagtgatcacagacgccgtggccggactgcctcatgctgtgcgggtgtccgccagagactttctggatgccggcacctggtctacctggtccccagaagcctggggcacaccttctactggcggacctgctggacagtctggcggaggcggaggaagtggcggaggatcagggggaggatctgtgcctggacctcctccaggaccccctagagtgtccccagatcctagggccgagctggactctaccgtgctgctgaccagatccctgctggccgacacaaggcagctggctgcccagctgagagacaagttccccgccgacggcgaccacaacctggatagcctgcctaccctggccatgtctgctggcgcactgggggctctgcagctgcctggggtgctgactagactgagagccgacctgctgagctacctgcggcatgtgcagtggctgagaagggctggcggcagcagcctgaaaaccctggaacctgagctgggcacactgcaggccagactggacagactgctgcgcagactgcagctgctgatgagcagactggctctgccccagcctcctcctgaccctcctgctcctccactggctcctccaagctctgcttggggcggaattagagccgcccacgccattctgggaggcctgcacctgacactggattgggcagtgcggggcctgctgctgctgaaaaccagactgcaccaccaccatcaccactgataagctt

SEQ ID NO: 99 - protein, 516 aa, Artificial Sequence
  IL-11:IL-11Ralpha fusion protein
MGWSCIILFLVATATGVHSPQAWGPPGVQYGQPGRSVKLCCPGVTAGDPVSWFRDGEPKLLQGPDSGLGHELVLAQADSTDEGTYICQTLDGALGGTVTLQLGYPPARPVVSCQAADYENFSCTWSPSQISGLPTRYLTSYRKKTVLGADSQRRSPSTGPWPCPQDPLGAARCVVHGAEFWSQYRINVTEVNPLGASTRLLDVSLQSILRPDPPQGLRVESVPGYPRRLRASWTYPASWPCQPHFLLKFRLQYRPAQHPAWSTVEPAGLEEVITDAVAGLPHAVRVSARDFLDAGTWSTWSPEAWGTPSTGGPAGQSGGGGGSGGGSGGGSVPGPPPGPPRVSPDPRAELDSTVLLTRSLLADTRQLAAQLRDKFPADGDHNLDSLPTLAMSAGALGALQLPGVLTRLRADLLSYLRHVQWLRRAGGSSLKTLEPELGTLQARLDRLLRRLQLLMSRLALPQPPPDPPAPPLAPPSSAWGGIRAAHAILGGLHLTLDWAVRGLLLLKTRLHHHHHH